European Patent Application EP 4 324 928 A1, published February 21, 2024. Title: Synthetic reagents for enzyme-catalysed alkylation. Applicant: Universität Basel. The sequence listing filed with the application follows.

SEQUENCE LISTING (1 sequence)

SEQ ID NO: 1 - protein, 207 aa, unidentified
  VARIANT 23: note = X can be Trp, Tyr or Phe
  VARIANT 34: note = X can be Trp, Tyr or Phe
  VARIANT 59: note = X can be Gly
  VARIANT 61: note = X can be Gly
  VARIANT 80: note = X can be Asp or Glu
  VARIANT 122: note = X can be Ala, Ser or Thr
  VARIANT 126: note = X can be Gly, Ala, Ser or Thr
  VARIANT 163: note = X can be Ala, Pro, Ser
MSDPTQPAVPDFETRDPNSPAFXDERFERRFTPXDQAGVPAAFQSFAARHSGAAVLIPXCXSAYEAVWLAGQGNPVRAIXFSPAAVAAAHEQLGAQHAQLVEQADFFTYEPPFTPAWIYERXFLCXLPLARRADYAHRMADLLPGGALLAGFFFLGATPKGPXFGIERAELDALLTPYFDLIEDEAVHDSIAVFAGRERWLTWRRRA